European Patent Application EP 4 681 781 A2, published January 21, 2026. Title: Centro De Ingenieria Genetica Y Biotecnologia. Applicant: Centro De Ingenieria Genetica Y Biotecnologia. Application EP. The sequence listing filed with the application follows.

SEQUENCE LISTING (9 sequences)

SEQ ID NO: 1 - protein, 25 aa, synthetic construct
GRKKRRQRRRPPQACWMSPRHLGTC

SEQ ID NO: 2 - DNA, 20 bp, Homo sapiens
  source 1..20: mol_type = genomic DNA
ccaatgcatggccctcttct

SEQ ID NO: 3 - DNA, 22 bp, Homo sapiens
  source 1..22: mol_type = genomic DNA
gggttcctctacagctttccta

SEQ ID NO: 4 - DNA, 22 bp, Homo sapiens
  source 1..22: mol_type = genomic DNA
gtccaccaccctgttgctgtag

SEQ ID NO: 5 - DNA, 22 bp, Homo sapiens
  source 1..22: mol_type = genomic DNA
acttcaacagcgacacccactc

SEQ ID NO: 6 - DNA, 22 bp, Homo sapiens
  source 1..22: mol_type = genomic DNA
tagaggtcacaactgcccgaag

SEQ ID NO: 7 - DNA, 22 bp, Homo sapiens
  source 1..22: mol_type = genomic DNA
ggccatccctgagcttgaatag

SEQ ID NO: 8 - DNA, 22 bp, Homo sapiens
  source 1..22: mol_type = genomic DNA
acgtctgggcatttggagtatt

SEQ ID NO: 9 - DNA, 22 bp, Homo sapiens
  source 1..22: mol_type = genomic DNA
ctccatgcggtagtccttctct